European Patent Application EP 4 350 002 A1, published April 10, 2024. Title: Detection of molecular analytes based on prearranged probe competition. Applicant: Biotype GmbH. The sequence listing filed with the application follows.

SEQUENCE LISTING (23 sequences)

SEQ ID NO: 1 - DNA, 149 bp, Homo sapiens
  source 1..149: mol_type = genomic DNA
  gene 1..149: gene = Epidermal Growth Factor Receptor; gene_synonym = EGFR, COSG150 (GRCh38, 7:55019101..55211628
ctctctgtcatagggactctggatcccagaaggtgagaaagttaaaattcccgtcgctatcaaggaattaagagaagcaacatctccgaaacccaacaaggaaatcctcgatgtgagtttctgctttgctgtgtgggggtccatggctc

SEQ ID NO: 2 - DNA, 149 bp, synthetic construct
  source 1..149: mol_type = other DNA
  misc_feature 68: note = T>G SNP
ctctctgtcatagggactctggatcccagaaggtgagaaagttaaaattcccgtcgctatcaaggaagtaagagaagcaacatctccgaaacccaacaaggaaatcctcgatgtgagtttctgctttgctgtgtgggggtccatggctc

SEQ ID NO: 3 - DNA, 148 bp, synthetic construct
  source 1..148: mol_type = other DNA
  misc_feature 67: note = (A) deletion 1 nt
ctctctgtcatagggactctggatcccagaaggtgagaaagttaaaattcccgtcgctatcaaggattaagagaagcaacatctccgaaacccaacaaggaaatcctcgatgtgagtttctgctttgctgtgtgggggtccatggctc

SEQ ID NO: 4 - DNA, 147 bp, synthetic construct
  source 1..147: mol_type = other DNA
  misc_feature 67..68: note = (AT) deletion 2nt
ctctctgtcatagggactctggatcccagaaggtgagaaagttaaaattcccgtcgctatcaaggataagagaagcaacatctccgaaacccaacaaggaaatcctcgatgtgagtttctgctttgctgtgtgggggtccatggctc

SEQ ID NO: 5 - DNA, 140 bp, Homo sapiens
  source 1..140: mol_type = genomic DNA
  misc_feature 67..77: note = Deletion 11nt
  misc_feature 76..77: note = (GC) insertion
  gene 1..140: gene = Epidermal Growth Factor Receptor; gene_synonym = EGFR, COSM12422 (GRCh38, 7:55174775..55174785)
ctctctgtcatagggactctggatcccagaaggtgagaaagttaaaattcccgtcgctatcaaggagccaacatctccgaaacccaacaaggaaatcctcgatgtgagtttctgctttgctgtgtgggggtccatggctc

SEQ ID NO: 6 - DNA, 17 bp, synthetic construct
  source 1..17: mol_type = other DNA
  primer_bind 1..17: note = binds to location 1..17 on T1-w
ggatcccagaaggtgag

SEQ ID NO: 7 - DNA, 19 bp, synthetic construct
  source 1..19: mol_type = other DNA
  primer_bind 1: note = binds to location 130..149 on T1-w
atcgaggatttccttgttg

SEQ ID NO: 8 - DNA, 18 bp, synthetic construct
  source 1..18: mol_type = other DNA
  misc_feature 1: note = 6-FAM, 6-carboxylfluorescein
  misc_feature 18: note = TQ2, Tide Quencher
aattcccgtcgctatcaa

SEQ ID NO: 9 - DNA, 28 bp, synthetic construct
  source 1..28: mol_type = other DNA
  misc_feature 28: note = TQ2, Tide Quencher
  misc_feature 1: note = HEX, 2,4,5,7,1,4-hexa chlorofluorescein
cgtcgctatcaaggaattaagagaagca

SEQ ID NO: 10 - DNA, 18 bp, synthetic construct
  source 1..18: mol_type = other DNA
  misc_feature 1: note = 6-FAM (hexanyl)
  misc_feature 18: note = 3-blocker, C3: pronanyl alkyl alcohol
  misc_feature 2: note = locked nucleic acid (A), LNA (+A)
aattcccgtcgctatcaa

SEQ ID NO: 11 - DNA, 28 bp, synthetic construct
  source 1..28: mol_type = other DNA
  misc_feature 1: note = 6-FAM (CuAAC)
  misc_feature 28: note = 3-blocker, C3: pronanyl alkyl alcohol
  misc_feature 2: note = Locked nucleic acid (G), LNA (+G)
cgtcgctatcaaggaattaagagaagca

SEQ ID NO: 12 - DNA, 24 bp, synthetic construct
  source 1..24: mol_type = other DNA
  misc_feature 1: note = 6-FAM
  misc_feature 24: note = TQ2, Tide Quencher
  misc_feature 2: note = Locked nucleic acid (A), LNA (+A)
taaaattcccgtcgctatcaagga

SEQ ID NO: 13 - DNA, 25 bp, unidentified
  source 1..25: mol_type = other DNA
  misc_feature 1: note = HEX
  misc_feature 14: note = Locked nucleic acid (T), LNA (+T)
  misc_feature 25: note = TQ2, Tide Quencher
  misc_feature 2: note = Locked nucleic acid (G), LNA (+G)
cgctatcaaggaattaagagaagca

SEQ ID NO: 14 - DNA, 24 bp, synthetic construct
  source 1..24: mol_type = other DNA
  misc_feature 1: note = 6-FAM (hexanyl)
  misc_feature 24: note = 3-blocker C3: pronanyl alkyl alcohol
  misc_feature 2: note = Locked nucleic acid (A), LNA (+A)
taaaattcccgtcgctatcaagga

SEQ ID NO: 15 - DNA, 25 bp, synthetic construct
  source 1..25: mol_type = other DNA
  misc_feature 1: note = 6-FAM (CuAAC)
  misc_feature 14: note = Locked nucleic acid (T), LNA (+T)
  misc_feature 25: note = 3-blocker C3: pronanyl alkyl alcohol
  misc_feature 2: note = Locked nuleic acid (G), LNA (+G)
cgctatcaaggaattaagagaagca

SEQ ID NO: 16 - DNA, 24 bp, synthetic construct
  source 1..24: mol_type = other DNA
  misc_feature 1: note = 6-FAM (hexanyl)
  misc_feature 24: note = TQ2, Tide Quencher
  misc_difference 2: note = Locked nucleic acid (A), LNA (+A)
taaaattcccgtcgctatcaagga

SEQ ID NO: 17 - DNA, 25 bp, synthetic construct
  source 1..25: mol_type = other DNA
  misc_feature 1: note = Dy 631
  misc_feature 14: note = Locked nucleic acid (T), LNA (+T)
  misc_feature 25: note = TQ2, Tide Quencher
  misc_feature 2: note = Locked nucleic acid (G), LNA (+G)
cgctatcaaggaattaagagaagca

SEQ ID NO: 18 - DNA, 20 bp, synthetic construct
  source 1..20: mol_type = other DNA
  primer_bind 1..20: note = flanks variation COSM783 in GRCh38, 13:28018505..28018505
tcacggcacagcccagtaaa

SEQ ID NO: 19 - DNA, 21 bp, synthetic construct
  source 1..21: mol_type = other DNA
  primer_bind 1..21: note = flanks variation COSM783 in GRCh38, 13:28018505..28018505
aatagcagcctcacattgccc

SEQ ID NO: 20 - DNA, 29 bp, synthetic construct
  source 1..29: mol_type = other DNA
  primer_bind 1..29: note = flanks variations: COSM17559, COSM17571, COSM17572, COSM17573 in GRCh38, 5:171410543..171410544
atgtctatgaagtgttgtggttccttaac

SEQ ID NO: 21 - DNA, 24 bp, synthetic construct
  source 1..24: mol_type = other DNA
  primer_bind 1..24: note = flanks variations: COSM17559, COSM17571, COSM17572, COSM17573 in GRCh38, 5:171410543..171410544
acacggtagggaaagttctcactc

SEQ ID NO: 22 - DNA, 271 bp, Homo sapiens
  source 1..271: mol_type = genomic DNA
  gene 1..271: gene = fms-like tyrosine kinase 3; gene_synonym = FLT3, GRCh38, 13:28018453..28018723
tcacggcacagcccagtaaagataagaggccttccatcaccggtacctcctactgaagttgagtctagaagaaagattgcactccaggataatacacatcacagtaaataacactctggtgtcattcttgacagtgtgttcacagagacctggccgccaggaacgtgcttgtcacccacgggaaagtggtgaagatatgtgactttggattggctcgagatatcatgagtgattccaactatgttgtcaggggcaatgtgaggctgctatt

SEQ ID NO: 23 - DNA, 205 bp, Homo sapiens
  source 1..205: mol_type = genomic DNA
  gene 1..205: gene = Nucleophosmin 1; gene_synonym = NPM1, GRCh38, 5:171410473..171410677
atgtctatgaagtgttgtggttccttaaccacatttctttttttttttttccaggctattcaagatctctggcagtggaggaagtctctttaagaaaatagtttaaacaatttgttaaaaaattttccgtcttatttcatttctgtaacagttgatatctggctgtcctttttataatgcagagtgagaactttccctaccgtgt